European Patent Specification EP 3 607 073 B1, published June 5, 2024. Title: TISSUE SELECTIVE TRANSGENE EXPRESSION. Applicant: ENCODED GENOMICS, INC. The sequence listing filed with the application follows.

SEQUENCE LISTING (43 sequences)

SEQ ID NO: 1 - DNA, 681 bp, Homo sapiens
ggaggaagccatcaactaaactacaatgactgtaagatacaaaattgggaatggtaacatattttgaagttctgttgacataaagaatcatgatattaatgcccatggaaatgaaagggcgatcaacactatggtttgaaaagggggaaattgtagagcacagatgtgttcgtgtggcagtgtgctgtctctagcaatactcagagaagagagagaacaatgaaattctgattggccccagtgtgagcccagatgaggttcagctgccaactttctctttcacatcttatgaaagtcatttaagcacaactaactttttttttttttttttttttttgagacagagtcttgctctgttgcccaggacagagtgcagtagtgactcaatctcggctcactgcagcctccacctcctaggctcaaacggtcctcctgcatcagcctcccaagtagctggaattacaggagtggcccaccatgcccagctaatttttgtatttttaatagatacgggggtttcaccatatcacccaggctggtctcgaactcctggcctcaagtgatccacctgcctcggcctcccaaagtgctgggattataggcgtcagccactatgcccaacccgaccaaccttttttaaaataaatatttaaaaaattggtatttcacatatatactagt

SEQ ID NO: 2 - DNA, 502 bp, Mus musculus
agtttggacaagaactatagttctagctttctctgggtctccaccttgcagagaatgcagctttcattatctcatgagccaaactctcatcatctctttccatatatctgtcggtgctcttccatgagtactctaacacacacagaaggagcacttacacaggctgttgtttttctcttattatcatagctgttgttcagacatgtgcattctgttcttgttgcttcaatgctaaaggagtctcaggatatgagaactgtaccagccgaggcatcaggaaacatgggtggaaattcccacagtactatttgttcactgtgtgaccttgggccagtcacatccctttcctgaggcttcgattccccaagctataaaagaagcatctcttaacctttttttaggtcatgagtcaggcccagcacactctcagggagactcatgagagtacagatcatttcccatagaaaaaccatagttttatatccagaggcttttctgtaag

SEQ ID NO: 3 - DNA, 823 bp, Mus musculus
ggttccagttcagaggcagagcatttggggttcccagtcaggagctttcctctctccgctccttagtttcctctctttaaaaaaaaatgggtgatagtatagaaaggaagctctgggctcggggaccagggccctgggatccccgctcccagccactcgctcctgacccttccagggacaagctcccccccaccccgtcctttccaggctgccactagaagagatggggacgcgtggtcagccgcttctgtcgccccccagggaacggtctcacgctggagggggcagtgccctcggaacaggacagtcagcccaagccagccaagcgcgcgcggacgtccttcaccgcagagcaattgcaggtaccccgggcaagccccgaagcgtgtgggcggggcttcggagtgggcgtggttgttcgggacttgtgactccgccccttgtgcggggacccgcgtgaggccgctccaaggatgaagctgcctggggcgtggcctcggaccctgagcctctgattgggcggaggtctcagggcccttctgcgccccacaggttatgcaggcgcagttcgcgcaggacaacaacccggacgcgcagacgctgcagaagctggcggacatgacgggcctcagtcgcagggtcatccaggtggggctccggggtctcggccttcaggtctagggtgaaccttagggaagcgctgaagctcgtagtggtacggatggtcgcgcgtgcacgtggccgcccctctccagtgtggcctaaggaccccagtcggcacgggttgacccttttccttgattactgagagtgcagaggctgt

SEQ ID NO: 4 - DNA, 633 bp, Mus musculus
tggtgggaagacatgtccagggaagaaatggcctccagaggcctgaggtggggaaatgctggaggtggagagaggaacaactgactgaaaatgagcttccactgtggcttagtagcctataccaagtctagagtatagggtaggagaagattaggaaagcgatgggtctgagaatgatgtggcctgttgacttttgtaaacccaaagcaccttggactaaaccctatgaacagtgtggtgccaccaaagactataatgagctcagggaacagaattctgtgtgcatggtgattttttttttttttttctgctaactgcagtctgggtgatgcattgacaaaccaatcctggaaagtaagaggcaagggcagctgggacggtgagaggagcctgatgggaaccaggccaagcagggcagcagaggcgatgaagaggatgtggtgcatccagagactcacttcattagctggaggcactgctggatagggtctgaaggttctggtatctgagttggcgggctgggtgagtggtggctctgcttcctgaacagtgtgtgcaagaggaaacagggttaagggctaggacagtcacaggtgagtcagcctcacaagagcaaccttcccctagtgcaga

SEQ ID NO: 5 - DNA, 670 bp, Mus musculus
ggaggtctccttttgccccggttccaacaagagaatgcaaggctgtatctcaatttccttgagcctctctgtattatagaagaaaagtagggaagccatacgccccttctgagcttcagtgtctctctgtctctgcaaatgaggctggggaggctgggggcgggcgtgaaagaggcccgcgccaagccgacccccacctctgccccctccccaggtcaacaacctcatctggcacgtgcggtgcctcgagtgctccgtgtgtcgcacatcgctgaggcagcagaatagctgctacatcaagaacaaggagatctactgcaagatggactacttcaggtaggcagcggccatcccgccagcaagcgctggagcatgaacgccttgcacacgcgtgcctaggccacttgtgtggcctgtgctctccaattcctgagccctgctgttcagagtgcacaacgcggctcagcgcactggcccggccctcctactcagcacgtcttacacagaagggagcgccagtctcagcctgagttctggcgggggatctgcctcgggttcctccgatctgacaggcgctggccacgggtctggttccatctctggtcttttctggccccgagcaccagtgtgttctgttgagctctgatgtccgaggctctggcccggatca

SEQ ID NO: 6 - DNA, 1043 bp, Mus musculus
ctctggctacctcttatcttgggcattcacgacaatttctaattgcaggtagtttgtgtgtgtgcgcgtgttttttttccccctcagaggcttggattgcaaaggaactaagcgattacttcaagagccacgggttaagtgcagggagagggggagagagagggaaaaaaacccaatccaaattcaaattgcttcattagagagacaccgcttttgtggggaagggctttaaatgcccactacaaagttaggactcattgttcagcgccggtttatataacaggcgaggggaggcgctgggctctgacagctccgagccagttcagcagccgccgtcgcctgcattccctccccctcccccaggtgatggcccagccagggtccggctgcaaagcgaccacccgctgtctcgaagggaccgctccgcctgccatggtgagtcctttcggtcctgctttcggccccgagtccccccaacagcacaggccagggcttctggctcagccttccggctaccaacctctacccctgcgctggaaaactgccgataggagccgcctctcgttgagccttggtttttctggcctggaatgtgagctttggctgcttcctgcacccaggatgcgctgtgttaaaagttgggggccgtcccttcttctccaataggtcctttcattcttgtactccagcctagggcgcgacatccctggcacatttcggtgtcagtcggtgcgcgaggaaaccagattcaactctgagtactcggctaagcgcttcgctgttcctctctcccatttcaggctcagtcagacgcagaggccttggcaggcgctctggacaaggacgaaggtagagcctccccatgtacgcccagcacaccgtctgtctgctcgccgccctctgctgcctcttccgtgccgtctgccggcaagaatatctgctccagttgcggtctggagatcctggaccggtatctgctcaaggtgagtcagggtaggtgtgcctgcttgcccacgggtgtggtttgcagccccaagagctgt

SEQ ID NO: 7 - DNA, 507 bp, Mus musculus
caagacttttaaaagtttagataaataaacaaacatttgacggctttccatcacatctagactataatccaaagatctatatggtcccaaacgacttacacttaactaccgtctcccatatggcttcttcccccatcagtcattgtcctcagccatagtggcctccctgttcctttgggtacaagggaacaactccctgagaggttccattagctgctgttgcctgagatgctcttgagcccacaccatctgctcatttctctcctcacgtgtcagtgattaagaggctgtccttggcctcccgtcaaaattacatccctgccgctttccacttcttgccttcttattttctaaatagaactaactcaccactacccaacattctatataattggatatctgtcctctgtttaaatataatgttgacttcaagaaagaacgttgtcactgccctgtcaccagacttttaaacagtgcctatcgtgtggcacatgctcagtgaaattg

SEQ ID NO: 8 - DNA, 502 bp, Mus musculus
tcaacagggggacacttgggaaagaaggatggggacagagccgagaggactgttacacattagagaaacatcagtgactgtgccagctttggggtagactgcacaaaagccctgaggcagcacaggcaggatccagtctgctggtcccaggaagctaaccgtctcagacagagcacaaagcaccgagacatgtgccacaaggcttgtgtagagaggtcagaggacagcgtacaggtcccagagatcaaactcaacctcaccaggcttggcagcaagcctttaccaacccacccccaccccacccaccctgcacgcgcccctctcccctccccatggtctcccatggctatctcacttggccctaaaatgtttaaggatgacactggctgctgagtggaaatgagacagcagaagtcaacagtagattttaggaaagccagagaaaaaggcttgtgctgtttttagaaagccaagggacaagctaagatagggcccaagtaat

SEQ ID NO: 9 - DNA, 788 bp, Mus musculus
aaatagaactgtgagatagggggagagggggcaggaaggacaagagacccctgtctcattgtgatccccacctgtctgctctgtgggagggtacccatgagggccagcccacagcccttaggtggacattgtctggtcctgtctcactgtccctcccagcagccccagaggccaggagacaggggtctcagtcctcactgagagatgtgtaaactgaggcccagtgaatgttgagggccagggcatgcccttggtgggatgtgacctgggtctccttcgcacgggcttcctccccgaagccgagctgagcatttggagtttgaaatgtttccgtacttagcaatctgctcctctattcccgggcggacttccgatagctccggccttatgctgcactagataagatggagcagggagaggacacggcactacttatgtaaccggcctcttgaaaaatggagcagcggtcagggcggaacaagacgtcctctctctacgcatccctctcctttccctgctaaggctgcagctggagtcagaggcagggctgttccaatctgtctttgatcagtaacgcagccagcctccagcctccgtcagcctcctcatggctgagacccggcctcagtttcccccacttacatcccgaggatcagagcctgtgaggatgaaatgggataaggtagctggaaccgtctggcagagagcgagtcctcaggactgttgatgcctgtggctgcctggcttgaccccaagtgaccccgcctcctcatcctgcagcaggagaa

SEQ ID NO: 10 - DNA, 502 bp, Mus musculus
tctatagaatgtgtccccagccttgttttccacacttgatacgcaaggaatgcataccacagagagggatgagggtagcatccagcctgcttcctgtgtgtcggggcgctacagccacatctccccagtccatctcagaccgtcacagagcttcgccgaatgtatagctttgttctctgtgcagacagggagacagagccttgggaagcataggtgcttgcttctttgcccactgagtcttagctggacttgcacaccacatgcctcacagccgggcgcacttgcatttgtcacccaggcccagtgatgatggctctgcttgctttgtgctttgtgccaactacagctccagcacctgtgccctgggttttcactcctttagttgaacacgtagttactggggttgtagggatggagcctttctgcttccttctggcaaagtccttagcggcctgctgcgggggtggggggtgttcaggggagtggtgatgaagtatgacag

SEQ ID NO: 11 - DNA, 533 bp, Mus musculus
tctccagttggagaaacagatgctgtaactggggccacagtataaagagagcccagacattgaactgtcaacacagaagcctggcacactggaactggcagtccagctgggaacaaggggtagaggctgaggccactaagtcaactgaggcaggagacataggagctaaagcagctgaagggtgcaggacagctggggggtctgaagtgggcctcatgcccagagctatgaagtcaggggctgtagcctaggagccttggaagccagctggcaagctgtggcccaaagacgctgactcaccaggagggggcagctggagccaggcactcctaaggtttccaggaagggcagccttccagggctcagctaggggagacagtgttgacagcaagttgtcaggcaacttgagctactgggcagctgggaagctgtcccttggtccccagtatcatcatcaccccagacgctgcccacctgcctcaggtcccacacagtgatcctcccatctttaacacaacacatgaccagagaga

SEQ ID NO: 12 - DNA, 524 bp, Mus musculus
gtcaccctccccccaaacaaccccttcttctctggttcgagaaattacaggcatgaaagatataaatcgggatgcttgacttgggaatataaatcactaaagcttgggggcaggggtgggcgacctttgtgaccgtccttgtgcgtgccagtaaatcctgtggtccaggggagaagaaaaggctgtgtggcttctgctcacaaagctgcagaaaccattctttaagcccaaaagcacttccagagagagcagagcatccccaggctgctggctcagcaagttcactgtgctcaatctcaggaagtgaggataagagcagtgcctggagagtgcctggtgctgagctgagggtttctgaacacattaaagcggggagcatggaccgggcctcaggaggggtgttgaacatccctaggcagaggagtctagcttcctgggaaaagatatcaggttaagcacacacatgtcctctggaataagataatctttctgatcacacactatacacacacaaaagcctgctc

SEQ ID NO: 13 - DNA, 509 bp, Mus musculus
gccctctaggccacctgaccaggtcccctcagtcccccccttcccacactcccacactcagcccccctcccccccccccgacccctgcaggattatcctgtctgtgttcctgactcagcctgggagccacctgggcagcaggggccaagggtgtcctagaagggacctggagtccacgctgggccaagcctgccctttctccctctgtcttccgtccctgcttgcggttctgctgaatgtggttatttctctggctccttttacagagaatgctgctgctaattttatgtggagctctgaggcagtgtaattggaagccagacaccctgtcagcagtgggctcccgtcctgagctgccatgcttcctgctctcctcccgtcccggctcctcatttcatgcagccacctgtcccagggagagaggagtcacccaggcccctcagtccgccccttaaataagaaagcctccgttgctcggcacacataccaagcagccgctggtgcaatct

SEQ ID NO: 14 - DNA, 398 bp, Mus musculus
gtgttcttcccttcccctttggacccccgagacaagccaataaaatactcggcagggtggcttctctcctttttttgccagtaataaacagactcagagcaagttaagggtctggtccaaggtcatggctgggatcagtgacagagcccagaagagaacctgagacttcttgctgagccaagctggagaggacagaaaggaatgcgtctactccatgcatgaccctctgccagctttgctccttcctaagggaccatgaacgatatgtgcacaccgctcatacgtatgtgcacacctgcaagaggaggcatcccatgtacacctatgagacgcacagagaaacatatatgtagccataggctagaaattctttctctttctaggtctgcccctctgca

SEQ ID NO: 15 - DNA, 810 bp, Mus musculus
ggaccactcagtgtacacggaatgtagaattgagtctgccattggtcttccctcaaagtcttggaggcttgggactgatattgggagcatctgggcagagaaggccacaaagacagggtggtttttctacactgggacatactcgtgagcatgcacagaggcgtgtccccaacttccctgtcacccctgtcctctgccggctagaggggatgcgggggtggacatatgctgctattgggcagatatcacatgttaagaggtgggggggggctcaagaggcggagggctaggagcatcccatggggagaggttctggttttcttgctgcctctagctgctataaatacgttagcacttgagcaactggaaagctctgagtaatttaggatgcacaaagctgtaatttaactccagcatctcagtgtgcgagagcattaaagatgtaattaagatgtttacacaaagagattggagtctgtgacacttggggtgcaaaaccccaggaagggacacaatgggtgaggtgaggatctgtgggaggcctggggacagtcacttggatcccagctatgagatggcaggccacccagctgtttctccttggaaatgttttggcctgggggttgggggtggggcatcacactttgatatggagatggggcaacaaagcctgcaatatctgggggtggagaggtcaagtggatggagtcttttgagatcatgtcaggaagagggctcgatcccccaaaatcatggtgacatatggtgtctcggggttcacaggagctatgtctaaaatacaaaagtaaa

SEQ ID NO: 16 - DNA, 202 bp, Mus musculus
tctgcagaagcctgccattccaccatttaaacctgtgactccaggccttaagcctgttgaaggtcgagtcccagaagggtcatatgtgcaactgcctagggagagttcccactcgcagggccaagaggagtcccccggtctgaggtgtgggggcggggacgtgcactgggcgctgggaccacggctggggctcaggactcgc

SEQ ID NO: 17 - DNA, 937 bp, Mus musculus
tgcctcagtttcttcgcctagaaagccgggtctaagggtacatgccctgattcttttctggggtgtctcgaattttaaacaacacatactgttctgggctgatgacaagaggaagtactggtcggtggctgatggacatccaccatggtggcaactggagggagggggaacggacgttgaaaccctgccctcctggaatctgtcgcatgcacgcacgttgacaatgcttggcactggggacaggctgggatggatggagcggagcgtgaggaggagtgggcatgcaggcccgagtgtctgttttgctgattgctccttttgctttcaaggagattaaactatttttagtccatgcctactgctggtgagacgctggaggaagcctttccatcgttgagattttctggaagctgccaagtgtggtcttcagctcaattctgggagcctcccagagtgggagggaggaacatttccatctgggggcttcggggacaggctaagatcttccctggggtccttgctgcgctggcctcctcaaaccacgctgcctcggcctgcataaagcagtaatctgatgtgcccgatgtttgtaacgctgtgtttaaaaaaagtaatttattttctaattattccttgtcttgcataaccatgcattgccaaagtgtcgctatttaaaatatttatctctccacgccgcaggagcagctctggagcgtggagggggaagaaataaaagtccgcgtgccagtcgcaggcatattactttgactcgtcctggtggctttgacgtctccctgtaaatacatttatttttcattaggacgtttctgagcttgtggcccccggagagcggagtgattacgctgttcatctgcaagcgatgcaatagaggggtactcgcagaatgacttccgcccagagcatcctgcgcctgtct

SEQ ID NO: 18 - DNA, 922 bp, Mus musculus
taaaataccttatttttttccagtctctaaactgctaatctcccaggctaagggattctgggacaaaggcaaggcctggaagtggaaatctgtaaaattagcttcagcggtattagtgtttgcagttgaagattgaaaaactgctttcccagggcctgattggaggctccactctcctccaggaagaggcaaggactctgggctggcactgaggacaaatcctgggaggctgctatggggcctgggagccaggctgccttgtgctagaggcctagagagtgtctgtgtcccaagtcccaagctacccccagcagctaacagcttttccagttctcaggcacagcaggtgccaagatcacgctctggagtccagctgggccccttcctcttctttttttttttttttttttaagacctcctggacactgttcctctccccccccccgtgaccccccccctcagttctcaaacacgtgagggttgggggagggttccacagccagagagaggggccagctctggtgcctgtgggtacgcccgcccgtatggcccatcaggcctcttgtgtgcttgattgcctctgattggctgcagctgaattcagcaaaagctattatttgcccttgatgagccaatcagatggcctcattggccattcagagcaggcaccggaacctgagggtggggtggggggtgggggatggagatgggactcagtgagggggtgggaagctctaaaacagatgcaggacctgagcctgtctgtgtccaccacgaccttcacacaggtcacacccccttcccctgacttgtcaccccaaaccagggcttgttgcccaaccccacctcacaattccctcactctgtaacacctttccatatacctctgcatgtctaaacccaagacttgctctatgaaatc

SEQ ID NO: 19 - DNA, 639 bp, Mus musculus
agaccctgcttagcacagctcttagcgggtcctttagggggtctcccagcgggcccagtgggaatgagataaggaaggacacagctgtccattctcccgtgcctgctaaggaggaaatggggccgccttacataattggggcaatttgttccactcttgtcctcctggtatcatggctatcaccccctccttgctcagggagtccttgattgagcgagaagctcaggcctccctctctccctcctgctgggggttgctgaacagagggtgtaggagccataggctctgtcactgctgagatctgccagatgtctaggccaggagaaaatggaaagggctaagtcacagcatatgtggccactcaggcctatagccccaaatctgcctggtaacccattatgtccccagagaatttgcatgggcggacaccctcatgccgggtctcagtaagggaaggggtgggaggcaaaaatatccctccccaccctgaatctccaccccctccccccagaaactgacacttggccttgtctaaggatgggttttcccaaaatccttctgaaaaaaacagaatttcaagagtcactccctccgggtctcagcctagaacatatgcagtatcccctgacgtccataggg

SEQ ID NO: 20 - DNA, 716 bp, Mus musculus
aaactggcacagtaatggcgggctgacagacaagggagtctgtagcacccgctgcctccgcccaccccttctccgagcaattaaaaggtgtttatgtggggctggcagtggcttctgcctcccttccattacgaacattaagagatcttgacccttccactttccccgctcttgaaaggagctgcagacacgtggagccaattaggcgcacgcgtgggcgccaagggcctgagcagctttttctccctgattgcggcgtttacagctgattattctcccctcacccaaacagtgctgcttcctggcaaggtgccacccagaggagccggctgggggcccctggggacaggggaggactggattagtaaatgggcatctatcgaatggctttcatatgtgtggctggaagggagaagggtagggccaggaatggtggcagcaagggcccaggtagcaatgagggttcttctaacccaccatttagggatagcgatcagaaaagggccctcgaggaggtgacctaaatgtgtgtagaagctgacggccactacacacacacacacacacacacacacacatacacaagcatccttgtccttggagtcggtcagcatgagcaagagaaagatgttcccagtggccatgagagtggagccctcctccctacttacatccaggttggatggccaggagatcctgagatccttcaagactcc

SEQ ID NO: 21 - DNA, 147 bp, Mus musculus
aagccacatcctgggtggaaatatatggcttcaattcccactcttccggatgacctctgtggggagccctggcttcaccttggtccagcttcatcccttagcctcgctgccaggaaggcagtgaggtcagaggctggtgctggcgtg

SEQ ID NO: 22 - DNA, 297 bp, Mus musculus
cctacctggtgcccgccaacatctgggggccatcctggccagcgccagcgtggtggtgaaggcactgtgcgccgtggtactgtttctctacctgctttccttcgctgtggacacgggctgcctggccgtcaccccaggctaccttttcccacccaacttctggatctggaccctggccacccacgggctcatggaacagcacgtgtgggacgtggccattagcctggccacagtggttgtggccgggcgattactggagcccctctggggagccttggagctgctcatcttcttctc

SEQ ID NO: 23 - DNA, 101 bp, Homo sapiens
aaacggacgggcctccgctgaaccagtgaggccccagacgtgcgcataaataacccctgcgtgctgcaccacctggggagagggggaggaccacggtaaat

SEQ ID NO: 24 - DNA, 101 bp, Homo sapiens
ggagcgagcgcatagcaaaagggacgcggggtccttttctctgccggtggcactgggtagctgtggccaggtgtggtactttgatggggcccagggctgga

SEQ ID NO: 25 - DNA, 101 bp, Homo sapiens
gctcaaggaagcgtcgcagggtcacagatctgggggaaccccggggaaaagcactgaggcaaaaccgccgctcgtctcctacaatatatgggagggggagg

SEQ ID NO: 26 - DNA, 547 bp, Homo sapiens
ttgagtacgttctggattactcataagaccttttttttttccttccgggcgcaaaaccgtgagctggatttataatcgccctataaagctccagaggcggtcaggcacctgcagaggagccccgccgctccgccgactagctgcccccgcgagcaacggcctcgtgatttccccgccgatccggtccccgcctccccactctgcccccgcctaccccggagccgtgcagccgcctctccgaatctctctcttctcctggcgctcgcgtgcgagagggaactagcgagaacgaggaagcagctggaggtgacgccgggcagattacgcctgtcagggccgagccgagcggatcgctgggcgctgtgcagaggaaaggcgggagtgcccggctcgctgtcgcagagccgaggtgggtaagctagcgaccacctggacttcccagcgcccaaccgtggcttttcagccaggtcctctcctcccgcggcttctcaaccaaccccatcccagcgccggccacccaacctcccgaaatgagtgcttcctgccc

SEQ ID NO: 27 - DNA, 101 bp, Homo sapiens
cagcagccgaaggcgctactaggaacggtaacctgttacttttccaggggccgtagtcgacccgctgcccgagttgctgtgcgactgcgcgcgcggggcta

SEQ ID NO: 28 - DNA, 201 bp, Homo sapiens
gagtgcaaggtgactgtggttcttctctggccaagtccgagggagaacgtaaagatatgggcctttttccccctctcaccttgtctcaccaaagtccctagtccccggagcagttagcctctttctttccagggaattagccagacacaacaacgggaaccagacaccgaaccagacatgcccgccccgtgcgccctcccc

SEQ ID NO: 29 - DNA, 199 bp, Homo sapiens
gctcgctgcctttcctccctcttgtctctccagagccggatcttcaaggggagcctccgtgcccccggctgctcagtccctccggtgtgcaggaccccggaagtcctccccgcacagctctcgcttctctttgcagcctgtttctgcgccggaccagtcgaggactctggacagtagaggccccgggacgaccgagctg

SEQ ID NO: 30 - DNA, 1351 bp, Homo sapiens
aaacggacgggcctccgctgaaccagtgaggccccagacgtgcgcataaataacccctgcgtgctgcaccacctggggagagggggaggaccacggtaaatggagcgagcgcatagcaaaagggacgcggggtccttttctctgccggtggcactgggtagctgtggccaggtgtggtactttgatggggcccagggctggagctcaaggaagcgtcgcagggtcacagatctgggggaaccccggggaaaagcactgaggcaaaaccgccgctcgtctcctacaatatatgggagggggaggttgagtacgttctggattactcataagaccttttttttttccttccgggcgcaaaaccgtgagctggatttataatcgccctataaagctccagaggcggtcaggcacctgcagaggagccccgccgctccgccgactagctgcccccgcgagcaacggcctcgtgatttccccgccgatccggtccccgcctccccactctgcccccgcctaccccggagccgtgcagccgcctctccgaatctctctcttctcctggcgctcgcgtgcgagagggaactagcgagaacgaggaagcagctggaggtgacgccgggcagattacgcctgtcagggccgagccgagcggatcgctgggcgctgtgcagaggaaaggcgggagtgcccggctcgctgtcgcagagccgaggtgggtaagctagcgaccacctggacttcccagcgcccaaccgtggcttttcagccaggtcctctcctcccgcggcttctcaaccaaccccatcccagcgccggccacccaacctcccgaaatgagtgcttcctgccccagcagccgaaggcgctactaggaacggtaacctgttacttttccaggggccgtagtcgacccgctgcccgagttgctgtgcgactgcgcgcgcggggctagagtgcaaggtgactgtggttcttctctggccaagtccgagggagaacgtaaagatatgggcctttttccccctctcaccttgtctcaccaaagtccctagtccccggagcagttagcctctttctttccagggaattagccagacacaacaacgggaaccagacaccgaaccagacatgcccgccccgtgcgccctccccgctcgctgcctttcctccctcttgtctctccagagccggatcttcaaggggagcctccgtgcccccggctgctcagtccctccggtgtgcaggaccccggaagtcctccccgcacagctctcgcttctctttgcagcctgtttctgcgccggaccagtcgaggactctggacagtagaggccccgggacgaccgagctg

SEQ ID NO: 31 - DNA, 2051 bp, Homo sapiens
ggaggaagccatcaactaaactacaatgactgtaagatacaaaattgggaatggtaacatattttgaagttctgttgacataaagaatcatgatattaatgcccatggaaatgaaagggcgatcaacactatggtttgaaaagggggaaattgtagagcacagatgtgttcgtgtggcagtgtgctgtctctagcaatactcagagaagagagagaacaatgaaattctgattggccccagtgtgagcccagatgaggttcagctgccaactttctctttcacatcttatgaaagtcatttaagcacaactaactttttttttttttttttttttttgagacagagtcttgctctgttgcccaggacagagtgcagtagtgactcaatctcggctcactgcagcctccacctcctaggctcaaacggtcctcctgcatcagcctcccaagtagctggaattacaggagtggcccaccatgcccagctaatttttgtatttttaatagatacgggggtttcaccatatcacccaggctggtctcgaactcctggcctcaagtgatccacctgcctcggcctcccaaagtgctgggattataggcgtcagccactatgcccaacccgaccaaccttttttaaaataaatatttaaaaaattggtatttcacatatatactagtatttacatttatccacacaaaacggacgggcctccgctgaaccagtgaggccccagacgtgcgcataaataacccctgcgtgctgcaccacctggggagagggggaggaccacggtaaatggagcgagcgcatagcaaaagggacgcggggtccttttctctgccggtggcactgggtagctgtggccaggtgtggtactttgatggggcccagggctggagctcaaggaagcgtcgcagggtcacagatctgggggaaccccggggaaaagcactgaggcaaaaccgccgctcgtctcctacaatatatgggagggggaggttgagtacgttctggattactcataagaccttttttttttccttccgggcgcaaaaccgtgagctggatttataatcgccctataaagctccagaggcggtcaggcacctgcagaggagccccgccgctccgccgactagctgcccccgcgagcaacggcctcgtgatttccccgccgatccggtccccgcctccccactctgcccccgcctaccccggagccgtgcagccgcctctccgaatctctctcttctcctggcgctcgcgtgcgagagggaactagcgagaacgaggaagcagctggaggtgacgccgggcagattacgcctgtcagggccgagccgagcggatcgctgggcgctgtgcagaggaaaggcgggagtgcccggctcgctgtcgcagagccgaggtgggtaagctagcgaccacctggacttcccagcgcccaaccgtggcttttcagccaggtcctctcctcccgcggcttctcaaccaaccccatcccagcgccggccacccaacctcccgaaatgagtgcttcctgccccagcagccgaaggcgctactaggaacggtaacctgttacttttccaggggccgtagtcgacccgctgcccgagttgctgtgcgactgcgcgcgcggggctagagtgcaaggtgactgtggttcttctctggccaagtccgagggagaacgtaaagatatgggcctttttccccctctcaccttgtctcaccaaagtccctagtccccggagcagttagcctctttctttccagggaattagccagacacaacaacgggaaccagacaccgaaccagacatgcccgccccgtgcgccctccccgctcgctgcctttcctccctcttgtctctccagagccggatcttcaaggggagcctccgtgcccccggctgctcagtccctccggtgtgcaggaccccggaagtcctccccgcacagctctcgcttctctttgcagcctgtttctgcgccggaccagtcgaggactctggacagtagaggccccgggacgaccgagctg

SEQ ID NO: 32 - DNA, 1878 bp, Unknown
  Description of Unknown: RE sequence
tcaacagggggacacttgggaaagaaggatggggacagagccgagaggactgttacacattagagaaacatcagtgactgtgccagctttggggtagactgcacaaaagccctgaggcagcacaggcaggatccagtctgctggtcccaggaagctaaccgtctcagacagagcacaaagcaccgagacatgtgccacaaggcttgtgtagagaggtcagaggacagcgtacaggtcccagagatcaaactcaacctcaccaggcttggcagcaagcctttaccaacccacccccaccccacccaccctgcacgcgcccctctcccctccccatggtctcccatggctatctcacttggccctaaaatgtttaaggatgacactggctgctgagtggaaatgagacagcagaagtcaacagtagattttaggaaagccagagaaaaaggcttgtgctgtttttagaaagccaagggacaagctaagatagggcccaagtaatgctagtatttacatttatccacacaaaacggacgggcctccgctgaaccagtgaggccccagacgtgcgcataaataacccctgcgtgctgcaccacctggggagagggggaggaccacggtaaatggagcgagcgcatagcaaaagggacgcggggtccttttctctgccggtggcactgggtagctgtggccaggtgtggtactttgatggggcccagggctggagctcaaggaagcgtcgcagggtcacagatctgggggaaccccggggaaaagcactgaggcaaaaccgccgctcgtctcctacaatatatgggagggggaggttgagtacgttctggattactcataagaccttttttttttccttccgggcgcaaaaccgtgagctggatttataatcgccctataaagctccagaggcggtcaggcacctgcagaggagccccgccgctccgccgactagctgcccccgcgagcaacggcctcgtgatttccccgccgatccggtccccgcctccccactctgcccccgcctaccccggagccgtgcagccgcctctccgaatctctctcttctcctggcgctcgcgtgcgagagggaactagcgagaacgaggaagcagctggaggtgacgccgggcagattacgcctgtcagggccgagccgagcggatcgctgggcgctgtgcagaggaaaggcgggagtgcccggctcgctgtcgcagagccgaggtgggtaagctagcgaccacctggacttcccagcgcccaaccgtggcttttcagccaggtcctctcctcccgcggcttctcaaccaaccccatcccagcgccggccacccaacctcccgaaatgagtgcttcctgccccagcagccgaaggcgctactaggaacggtaacctgttacttttccaggggccgtagtcgacccgctgcccgagttgctgtgcgactgcgcgcgcggggctagagtgcaaggtgactgtggttcttctctggccaagtccgagggagaacgtaaagatatgggcctttttccccctctcaccttgtctcaccaaagtccctagtccccggagcagttagcctctttctttccagggaattagccagacacaacaacgggaaccagacaccgaaccagacatgcccgccccgtgcgccctccccgctcgctgcctttcctccctcttgtctctccagagccggatcttcaaggggagcctccgtgcccccggctgctcagtccctccggtgtgcaggaccccggaagtcctccccgcacagctctcgcttctctttgcagcctgtttctgcgccggaccagtcgaggactctggacagtagaggccccgggacgaccgagctg

SEQ ID NO: 33 - DNA, 19 bp, Homo sapiens
atttacatttatccacaca

SEQ ID NO: 34 - DNA, 800 bp, Mus musculus
tgccgctggactctcttccaaggaactaggagaaccaagatccgtttttctgccaagggctgccccccccacgcccccaaccccctcaccccgatccccacagaaagaaatcttgaggtagctggagcttcttctgtgggtgtgacaggactgccattctcctctgtagtctgcagaagcctgccattccaccatttaaacctgtgactccaggccttaagcctgttgaaggtcgagtcccagaagggtcatatgtgcaactgcctagggagagttcccactcgcagggccaagaggagtcccccggtctgaggtgtgggggcggggacgtgcactgggcgctgggaccacggctggggctcaggactcgcgagcttggattcggatcggtttgcgcgagccagtagggcaggctccggggtgaacggggacgaggggcgcgcgggcacaggcgggcgcgtgaccgcggcgggggcgcgcggaggcgggccggccaaggagagggagggagggaatgagggagggagcgacaggggagggcggcgccggcaggttggcggcggccgctatttgagcgcaggtcccgggccaggcgctcaaagcgcttggagccagcgcggcggggagatcgctgcgcgcagcccgcagaggcgctgcggccagtgcagccccggaggccccgcgcggagaaggaggtggagaagaggccggctttccgcccgccgcccgcgcccccccacctccatcccgccgccgccgtcccccctccctccccgcggcgccgcatcttgaatggaaac

SEQ ID NO: 35 - DNA, 1335 bp, Artificial Sequence
  Description of Artificial Sequence: Synthetic polynucleotide
gagtaattcatacaaaaggactcgcccctgccttggggaatcccagggaccgtcgttaaactcccactaacgtagaacccagagatcgctgcgttcccgccccctcacccgcccgctctcgtcatcactgaggtggagaagagcatgcgtgaggctccggtgcccgtcagtgggcagagcgcacatcgcccacagtccccgagaagttggggggaggggtcggcaattgaaccggtgcctagagaaggtggcgcggggtaaactgggaaagtgatgtcgtgtactggctccgcctttttcccgagggtgggggagaaccgtatataagtgcagtagtcgccgtgaacgttctttttcgcaacgggtttgccgccagaacacaggtaagtgccgtgtgtggttcccgcgggcctggcctctttacgggttatggcccttgcgtgccttgaattacttccacgcccctggctgcagtacgtgattcttgatcccgagcttcgggttggaagtgggtgggagagttcgaggccttgcgcttaaggagccccttcgcctcgtgcttgagttgaggcctggcttgggcgctggggccgccgcgtgcgaatctggtggcaccttcgcgcctgtctcgctgctttcgataagtctctagccatttaaaatttttgatgacctgctgcgacgctttttttctggcaagatagtcttgtaaatgcgggccaagatctgcacactggtatttcggtttttggggccgcgggcggcgacggggcccgtgcgtcccagcgcacatgttcggcgaggcggggcctgcgagcgcggccaccgagaatcggacgggggtagtctcaagctggccggcctgctctggtgcctggcctcgcgccgccgtgtatcgccccgccctgggcggcaaggctggcccggtcggcaccagttgcgtgagcggaaagatggccgcttcccggccctgctgcagggagctcaaaatggaggacgcggcgctcgggagagcgggcgggtgagtcacccacacaaaggaaaagggcctttccgtcctcagccgtcgcttcatgtgactccacggagtaccgggcgccgtccaggcacctcgattagttctcgagcttttggagtacgtcgtctttaggttggggggaggggttttatgcgatggagtttccccacactgagtgggtggagactgaagttaggccagcttggcacttgatgtaattctccttggaatttgccctttttgagtttggatcttggttcattctcaagcctcagacagtggttcaaagtttttttcttccatttcaggtgtcgtga

SEQ ID NO: 36 - protein, 222 aa, Artificial Sequence
  Description of Artificial Sequence: Synthetic polypeptide
MVSKGEELFTGVVPILVELDGDVNGHKFSVSGEGEGDATYGKLTLKFICTTGKLPVPWPTLVTTLTYGVQCFSRYPDHMKQHDFFKSAMPEGYVQERTIFFKDDGNYKTRAEVKFEGDTLVNRIELKGIDFKEDGNILGHKLEYNYNSHNVYIMADKQKNGIKVNFKIRHNIEDGSVQLADHYQQNTPIGDGPVLLPDNHYLSTQSALSKDPNEKRDHMVLL

SEQ ID NO: 37 - protein, 218 aa, Unknown [sequence omitted]

SEQ ID NO: 38 - protein, 215 aa, Unknown
  Description of Unknown: SCN2B sequence
MHRDAWLPRPAFSLTGLSLFFSLVPPGRSMEVTVPATLNVLNGSDARLPCTFNSCYTVNHKQFSLNWTYQECNNCSEEMFLQFRMKIINLKLERFQDRVEFSGNPSKYDVSVMLRNVQPEDEGIYNCYIMNPPDRHRGHGKIHLQVLMEEPPERDSTVAVIVGASVGGFLAVVILVLMVVKCVRRKKEQKLSTDDLKTEEEGKTDGEGNPDDGAK

SEQ ID NO: 39 - protein, 2009 aa, Unknown
  Description of Unknown: SCN1A sequence
MEQTVLVPPGPDSFNFFTRESLAAIERRIAEEKAKNPKPDKKDDDENGPKPNSDLEAGKNLPFIYGDIPPEMVSEPLEDLDPYYINKKTFIVLNKGKAIFRFSATSALYILTPFNPLRKIAIKILVHSLFSMLIMCTILTNCVFMTMSNPPDWTKNVEYTFTGIYTFESLIKIIARGFCLEDFTFLRDPWNWLDFTVITFAYVTEFVDLGNVSALRTFRVLRALKTISVIPGLKTIVGALIQSVKKLSDVMILTVFCLSVFALIGLQLFMGNLRNKCIQWPPTNASLEEHSIEKNITVNYNGTLINETVFEFDWKSYIQDSRYHYFLEGFLDALLCGNSSDAGQCPEGYMCVKAGRNPNYGYTSFDTFSWAFLSLFRLMTQDFWENLYQLTLRAAGKTYMIFFVLVIFLGSFYLINLILAVVAMAYEEQNQATLEEAEQKEAEFQQMIEQLKKQQEAAQQAATATASEHSREPSAAGRLSDSSSEASKLSSKSAKERRNRRKKRKQKEQSGGEEKDEDEFQKSESEDSIRRKGFRFSIEGNRLTYEKRYSSPHQSLLSIRGSLFSPRRNSRTSLFSFRGRAKDVGSENDFADDEHSTFEDNESRRDSLFVPRRHGERRNSNLSQTSRSSRMLAVFPANGKMHSTVDCNGVVSLVGGPSVPTSPVGQLLPEVIIDKPATDDNGTTTETEMRKRRSSSFHVSMDFLEDPSQRQRAMSIASILTNTVEELEESRQKCPPCWYKFSNIFLIWDCSPYWLKVKHVVNLVVMDPFVDLAITICIVLNTLFMAMEHYPMTDHFNNVLTVGNLVFTGIFTAEMFLKIIAMDPYYYFQEGWNIFDGFIVTLSLVELGLANVEGLSVLRSFRLLRVFKLAKSWPTLNMLIKIIGNSVGALGNLTLVLAIIVFIFAVVGMQLFGKSYKDCVCKIASDCQLPRWHMNDFFHSFLIVFRVLCGEWIETMWDCMEVAGQAMCLTVFMMVMVIGNLVVLNLFLALLLSSFSADNLAATDDDNEMNNLQIAVDRMHKGVAYVKRKIYEFIQQSFIRKQKILDEIKPLDDLNNKKDSCMSNHTAEIGKDLDYLKDVNGTTSGIGTGSSVEKYIIDESDYMSFINNPSLTVTVPIAVGESDFENLNTEDFSSESDLEESKEKLNESSSSSEGSTVDIGAPVEEQPVVEPEETLEPEACFTEGCVQRFKCCQINVEEGRGKQWWNLRRTCFRIVEHNWFETFIVFMILLSSGALAFEDIYIDQRKTIKTMLEYADKVFTYIFILEMLLKWVAYGYQTYFTNAWCWLDFLIVDVSLVSLTANALGYSELGAIKSLRTLRALRPLRALSRFEGMRVVVNALLGAIPSIMNVLLVCLIFWLIFSIMGVNLFAGKFYHCINTTTGDRFDIEDVNNHTDCLKLIERNETARWKNVKVNFDNVGFGYLSLLQVATFKGWMDIMYAAVDSRNVELQPKYEESLYMYLYFVIFIIFGSFFTLNLFIGVIIDNFNQQKKKFGGQDIFMTEEQKKYYNAMKKLGSKKPQKPIPRPGNKFQGMVFDFVTRQVFDISIMILICLNMVTMMVETDDQSEYVTTILSRINLVFIVLFTGECVLKLISLRHYYFTIGWNIFDFVVVILSIVGMFLAELIEKYFVSPTLFRVIRLARIGRILRLIKGAKGIRTLLFALMMSLPALFNIGLLLFLVMFIYAIFGMSNFAYVKREVGIDDMFNFETFGNSMICLFQITTSAGWDGLLAPILNSKPPDCDPNKVNPGSSVKGDCGNPSVGIFFFVSYIIISFLVVVNMYIAVILENFSVATEESAEPLSEDDFEMFYEVWEKFDPDATQFMEFEKLSQFAAALEPPLNLPQPNKLQLIAMDLPMVSGDRIHCLDILFAFTKRVLGESGEMDALRIQMEERFMASNPSKVSYQPITTTLKRKQEEVSAVIIQRAYRRHLLKRTVKQASFTYNKNKIKGGANLLIKEDMIIDRINENSITEKTDLTMSTAACPPSYDRVTKPIVEKHEQEGKDEKAKGK

SEQ ID NO: 40 - protein, 603 aa, Unknown [sequence omitted]

SEQ ID NO: 41 - protein, 511 aa, Unknown
  Description of Unknown: Kv3.1 sequence
MGQGDESERIVINVGGTRHQTYRSTLRTLPGTRLAWLAEPDAHSHFDYDPRADEFFFDRHPGVFAHILNYYRTGKLHCPADVCGPLYEEELAFWGIDETDVEPCCWMTYRQHRDAEEALDSFGGAPLDNSADDADADGPGDSGDGEDELEMTKRLALSDSPDGRPGGFWRRWQPRIWALFEDPYSSRYARYVAFASLFFILVSITTFCLETHERFNPIVNKTEIENVRNGTQVRYYREAETEAFLTYIEGVCVVWFTFEFLMRVIFCPNKVEFIKNSLNIIDFVAILPFYLEVGLSGLSSKAAKDVLGFLRVVRFVRILRIFKLTRHFVGLRVLGHTLRASTNEFLLLIIFLALGVLIFATMIYYAERIGAQPNDPSASEHTHFKNIPIGFWWAVVTMTTLGYGDMYPQTWSGMLVGALCALAGVLTIAMPVPVIVNNFGMYYSLAMAKQKLPKKKKKHIPRPPQLGSPNYCKSVVNSPHHSTQSDTCPLAQEEILEINRAGRKPLRGMSI

SEQ ID NO: 42 - protein, 639 aa, Unknown
  Description of Unknown: Kv3.2 sequence
MGKIESNERVILNVGGTRHETYRSTLKTLPGTRLALLASSEPQGDCLTAAGDKLQPLPPPLSPPPRPPPLSPVPSGCFEGGAGNCSSHGGNGGNGGSDHPGGGREFFFDRHPGVFAYVLNYYRTGKLHCPADVCGPLFEEELAFWGIDETDVEPCCWMTYRQHRDAEEALDIFETPDLIGGDPGDDEDLAAKRLGIEDAAGLGGPDGKSGRWRKLQPRMWALFEDPYSSRAARFIAFASLFFILVSITTFCLETHEAFNIVKNKTEPVINGTSPVLQYEIETDPALTYVEGVCVVWFTFEFLVRIVFSPNKLEFIKNLLNIIDFVAILPFYLEVGLSGLSSKAAKDVLGFLRVVRFVRILRIFKLTRHFVGLRVLGHTLRASTNEFLLLIIFLALGVLIFATMIYYAERVGAQPNDPSASEHTQFKNIPIGFWWAVVTMTTLGYGDMYPQTWSGMLVGALCALAGVLTIAMPVPVIVNNFGMYYSLAMAKQKLPRKRKKHIPPAPLASSPTFCKTELNMACNSTQSDTCLGKENRLLEHNRSVLSGDDSTGSEPPLSPPERLPIRRSSTRDKNRRGETCFLLTTGDYTCASDGGIRKASTLEPMESTAQTKGDTRPEAHWNCAHLLNFGCPTGSSFPTL

SEQ ID NO: 43 - protein, 757 aa, Unknown
  Description of Unknown: Kv3.3 sequence
MLSSVCVSSFRGRQGASKQQPAPPPQPPESPPPPPLPPQQQQPAQPGPAASPAGPPAPRGPGDRRAEPCPGLPAAAMGRHGGGGGDSGKIVINVGGVRHETYRSTLRTLPGTRLAGLTEPEAAARFDYDPGADEFFFDRHPGVFAYVLNYYRTGKLHCPADVCGPLFEEELGFWGIDETDVEACCWMTYRQHRDAEEALDSFEAPDPAGAANAANAAGAHDGGLDDEAGAGGGGLDGAGGELKRLCFQDAGGGAGGPPGGAGGAGGTWWRRWQPRVWALFEDPYSSRAARYVAFASLFFILISITTFCLETHEGFIHISNKTVTQASPIPGAPPENITNVEVETEPFLTYVEGVCVVWFTFEFLMRITFCPDKVEFLKSSLNIIDCVAILPFYLEVGLSGLSSKAAKDVLGFLRVVRFVRILRIFKLTRHFVGLRVLGHTLRASTNEFLLLIIFLALGVLIFATMIYYAERIGADPDDILGSNHTYFKNIPIGFWWAVVTMTTLGYGDMYPKTWSGMLVGALCALAGVLTIAMPVPVIVNNFGMYYSLAMAKQKLPKKKNKHIPRPPQPGSPNYCKPDPPPPPPPHPHHGSGGISPPPPITPPSMGVTVAGAYPAGPHTHPGLLRGGAGGLGIMGLPPLPAPGEPCPLAQEEVIEINRADPRPNGDPAAAALAHEDCPAIDQPAMSPEDKSPITPGSRGRYSRDRACFLLTDYAPSPDGSIRKATGAPPLPPQDWRKPGPPSFLPDLNANAAAWISP